European Patent Application EP 4 257 598 A1, published October 11, 2023. Title: Fusion protein comprising glucagon like peptide-1 receptor agonist and anti-OSCAR antibody and uses thereof. Applicant: ImmunoForge Co.,Ltd. The sequence listing filed with the application follows.

SEQUENCE LISTING (10 sequences)

SEQ ID NO: 1 - protein, 116 aa, Artificial Sequence
  heavy chain of anti-OSCAR antibody
EVQLLESGGGLVQPGGSLRLSCAASGFTFSDYAMSWVRQAPGKGLEWVSGIYHGGGNIYYADSVKGRFTISRDNSKNTLYLQMNSLRAEDTAVYYCARAPDEFDYWGQGTLVTVSS

SEQ ID NO: 2 - protein, 110 aa, Artificial Sequence
  light chain of anti-OSCAR antibody
QSVLTQPPSASGTPGQRVTISCSGSSSNIGNNSVTWYQQLPGTAPKLLIYYNSHRPSGVPDRFSGSKPGTSASLAISGLRSEDEADYYCGAWDSSLNGYVFGGGTKLTVL

SEQ ID NO: 3 - protein, 118 aa, Artificial Sequence
  heavy chain of anti-OSCAR antibody
EVQLLESGGGLVQPGGSLRLSCAASGFTFSDYYWTWVRQAPGKGLEWVSGSPVFGAANYAQNFQGRFTISRDNSKNTLYLQMNSLRAEDTAVYYCAKAGFTGGHFDIWGQGTLVTVSS

SEQ ID NO: 4 - protein, 108 aa, Artificial Sequence
  light chain of anti-OSCAR antibody
QSVLTQPPSASGTPGQRVTISCSGSSSNIGNNYVSWYQQLPGTAPKLLIYGNSNRPSGVPNRFSGSKSGTSASLAISGLRSEDEADYYCQSYDSSSWLFGGGTKLTVL

SEQ ID NO: 5 - protein, 117 aa, Artificial Sequence
  heavy chain of anti-OSCAR antibody
EVQLLESGGGLVQPGGSLRLSCAASGFTFSDYYWTWVRQAPGKGLEWVSGSPVFGAANYAQNFQGRFTISRDNSKNTLYLQMNSLRAEDTAVYYCAKAGIPGHFDIWGQGTLVTVSS

SEQ ID NO: 6 - protein, 108 aa, Artificial Sequence; identical to SEQ ID NO: 4
  light chain of anti-OSCAR antibody

SEQ ID NO: 7 - protein, 519 aa, Artificial Sequence
  PF1803
HGEGTFTSDVSSYLEEQAAKEFIAWLVKGGGGSAPAPGGGGSDKTHTCPPCPAPELLGGPSVFLFPPKPKDTLMISRTPEVTCVVVDVSHEDPEVKFNWYVDGVEVHNAKTKPREEQYASTYRVVSVLTVLHQDWLNGKEYKCKVSNKALPAPIEKTISKAKGQPREPQVYTLPPSREEMTKNQVSLTCLVKGFYPSDIAVEWESNGQPENNYKTTPPVLDSDGSFFLYSKLTVDKSRWQQGNVFSCSVMHEALHNHYTQKSLSLSPGKGGGGSGGGGSEVQLLESGGGLVQPGGSLRLSCAASGFTFSDYYWTWVRQAPGKGLEWVSGSPVFGAANYAQNFQGRFTISRDNSKNTLYLQMNSLRAEDTAVYYCAKAGIPGHFDIWGQGTLVTVSSGGGGSGGGGSGGGGSQSVLTQPPSASGTPGQRVTISCSGSSSNIGNNYVSWYQQLPGTAPKLLIYGNSNRPSGVPNRFSGSKSGTSASLAISGLRSEDEADYYCQSYDSSSWLFGGGTKLTVL

SEQ ID NO: 8 - protein, 209 aa, Artificial Sequence
  Fc
SVFLFPPKPKDTLMISRTPEVTCVVVDVSHEDPEVKFNWYVDGVEVHNAKTKPREEQYNSTYRVVSVLTVLHQDWLNGKEYKCKVSNKALPAPIEKTISKAKGQPREPQVYTLPPSREEMTKNQVSLTCLVKGFYPSDIAVEWESNGQPENNYKTTPPVLDSDGSFFLYSKLTVDKSRWQQGNVFSCSVMHEALHNHYTQKSLSLSPGK

SEQ ID NO: 9 - protein, 209 aa, Artificial Sequence
  Fc N297A
SVFLFPPKPKDTLMISRTPEVTCVVVDVSHEDPEVKFNWYVDGVEVHNAKTKPREEQYASTYRVVSVLTVLHQDWLNGKEYKCKVSNKALPAPIEKTISKAKGQPREPQVYTLPPSREEMTKNQVSLTCLVKGFYPSDIAVEWESNGQPENNYKTTPPVLDSDGSFFLYSKLTVDKSRWQQGNVFSCSVMHEALHNHYTQKSLSLSPGK

SEQ ID NO: 10 - protein, 8 aa, Artificial Sequence
  OSC
GAGPAGFA